European Patent Application EP 4 686 762 A1, published February 4, 2026. Title: A method to characterize nucleic acid. Applicant: ICHORtec GmbH. Application EP, filed July 26, 2024. The sequence listing filed with the application follows.

SEQUENCE LISTING (7 sequences)

SEQ ID NO: 1 - DNA, 23 bp, synthetic construct
  source 1..23: mol_type = other DNA
agaccagaagatcaggaactcta

SEQ ID NO: 2 - DNA, 23 bp, synthetic construct
  source 1..23: mol_type = other DNA
tagagttcctgatcttctggtct

SEQ ID NO: 3 - DNA, 23 bp, synthetic construct
  source 1..23: mol_type = other DNA
tagagttcctgattttctggtct

SEQ ID NO: 4 - DNA, 40 bp, synthetic construct
  source 1..40: mol_type = other DNA
gtgagtttggggaaaaaaaataaaataaaaatggctttcc

SEQ ID NO: 5 - DNA, 40 bp, synthetic construct
  source 1..40: mol_type = other DNA
ggaaagccatttttattttattttttttccccaaactcac

SEQ ID NO: 6 - DNA, 40 bp, synthetic construct; identical to SEQ ID NO: 4
  source 1..40: mol_type = other DNA

SEQ ID NO: 7 - DNA, 40 bp, synthetic construct; identical to SEQ ID NO: 5
  source 1..40: mol_type = other DNA